European Patent Application EP 4 230 218 A1, published August 23, 2023. Title: Pharmaceutical composition for preventing or treating vasculitis comprising glucagon/GLP-1/GIP triple agonist or long acting conjugate thereof. Applicant: HANMI PHARM. CO., LTD. The sequence listing filed with the application follows.

SEQUENCE LISTING (138 sequences)

SEQ ID NO: 1 - protein, 30 aa, Artificial
  Triple agonist
  MISC_FEATURE (2)..(2): Xaa is aminoisobutyric acid (Aib)
HXQGTFTSDVSSYLDGQAAKEFIAWLVKGC

SEQ ID NO: 2 - protein, 30 aa, Artificial
  Triple agonist
  MISC_FEATURE (2)..(2): Xaa is aminoisobutyric acid (Aib)
HXQGTFTSDVSSYLDGQAQKEFIAWLVKGC

SEQ ID NO: 3 - protein, 41 aa, Artificial
  Triple agonist
  MISC_FEATURE (2)..(2): Xaa is aminoisobutyric acid (Aib)
HXQGTFTSDVSSYLLGQAAKQFIAWLVKGGGPSSGAPPPSC

SEQ ID NO: 4 - protein, 30 aa, Artificial
  Triple agonist
  MISC_FEATURE (2)..(2): Xaa is aminoisobutyric acid (Aib)
HXQGTFTSDVSSYLLGQQQKEFIAWLVKGC

SEQ ID NO: 5 - protein, 41 aa, Artificial
  Triple agonist
  MISC_FEATURE (2)..(2): Xaa is aminoisobutyric acid (Aib)
HXQGTFTSDVSSYLLGQQQKEFIAWLVKGGGPSSGAPPPSC

SEQ ID NO: 6 - protein, 30 aa, Artificial
  Triple agonist
  MISC_FEATURE (2)..(2): Xaa is aminoisobutyric acid (Aib)
HXQGTFTSDVSSYLDGQAAKEFVAWLLKGC

SEQ ID NO: 7 - protein, 30 aa, Artificial
  Triple agonist
  MISC_FEATURE (2)..(2): Xaa is aminoisobutyric acid (Aib)
HXQGTFTSDVSKYLDGQAAKEFVAWLLKGC

SEQ ID NO: 8 - protein, 30 aa, Artificial
  Triple agonist
  MISC_FEATURE (2)..(2): Xaa is aminoisobutyric acid (Aib)
HXQGTFTSDVSKYLDGQAAQEFVAWLLKGC

SEQ ID NO: 9 - protein, 30 aa, Artificial
  Triple agonist
  MISC_FEATURE (2)..(2): Xaa is aminoisobutyric acid (Aib)
HXQGTFTSDVSKYLDGQAAQEFVAWLLAGC

SEQ ID NO: 10 - protein, 41 aa, Artificial
  Triple agonist
  MISC_FEATURE (2)..(2): Xaa is aminoisobutyric acid (Aib)
HXQGTFTSDVSKYLDGQAAQEFVAWLLAGGGPSSGAPPPSC

SEQ ID NO: 11 - protein, 41 aa, Artificial
  Triple agonist
  MISC_FEATURE (1)..(1): Xaa is 4-imidazoacetyl (CA)
XGEGTFTSDLSKYLDSRRQQLFVQWLKAGGPSSGAPPPSHG

SEQ ID NO: 12 - protein, 41 aa, Artificial
  Triple agonist
  MISC_FEATURE (1)..(1): Xaa is 4-imidazoacetyl (CA)
XGEGTFISDLSKYMDEQAVQLFVEWLMAGGPSSGAPPPSHG

SEQ ID NO: 13 - protein, 41 aa, Artificial
  Triple agonist
  MISC_FEATURE (1)..(1): Xaa is 4-imidazoacetyl (CA)
XGEGTFISDYSIQLDEIAVQDFVEWLLAQKPSSGAPPPSHG

SEQ ID NO: 14 - protein, 41 aa, Artificial
  Triple agonist
  MISC_FEATURE (1)..(1): Xaa is 4-imidazoacetyl (CA)
XGQGTFTSDYSIQLDEIAVRDFVEWLKNGGPSSGAPPPSHG

SEQ ID NO: 15 - protein, 41 aa, Artificial
  Triple agonist
  MISC_FEATURE (1)..(1): Xaa is 4-imidazoacetyl (CA)
XGQGTFTSDLSKQMDEEAVRLFIEWLKNGGPSSGAPPPSHG

SEQ ID NO: 16 - protein, 41 aa, Artificial
  Triple agonist
  MISC_FEATURE (1)..(1): Xaa is 4-imidazoacetyl (CA)
XGQGTFTSDLSKQMDSEAQQLFIEWLKNGGPSSGAPPPSHG

SEQ ID NO: 17 - protein, 41 aa, Artificial
  Triple agonist
  MISC_FEATURE (1)..(1): Xaa is 4-imidazoacetyl (CA)
XGQGTFTSDLSKQMDEERAREFIEWLLAQKPSSGAPPPSHG

SEQ ID NO: 18 - protein, 41 aa, Artificial
  Triple agonist
  MISC_FEATURE (1)..(1): Xaa is 4-imidazoacetyl (CA)
XGQGTFTSDLSKQMDSERAREFIEWLKNTGPSSGAPPPSHG

SEQ ID NO: 19 - protein, 41 aa, Artificial
  Triple agonist
  MISC_FEATURE (1)..(1): Xaa is 4-imidazoacetyl (CA)
XGQGTFTSDLSIQYDSEHQRDFIEWLKDTGPSSGAPPPSHG

SEQ ID NO: 20 - protein, 41 aa, Artificial
  Triple agonist
  MISC_FEATURE (1)..(1): Xaa is 4-imidazoacetyl (CA)
XGQGTFTSDLSIQYEEEAQQDFVEWLKDTGPSSGAPPPSHG

SEQ ID NO: 21 - protein, 39 aa, Artificial
  Triple agonist
  MISC_FEATURE (2)..(2): Xaa is aminoisobutyric acid (Aib)
  MISC_FEATURE (16)..(20): amino acids at positions 16 and 20 form a ring
YXQGTFTSDYSKYLDECRAKEFVQWLLDHHPSSGQPPPS

SEQ ID NO: 22 - protein, 39 aa, Artificial
  Triple agonist
  MISC_FEATURE (2)..(2): Xaa is aminoisobutyric acid (Aib)
  MISC_FEATURE (16)..(20): amino acids at positions 16 and 20 form a ring
YXQGTFTSDYSKCLDEKRAKEFVQWLLDHHPSSGQPPPS

SEQ ID NO: 23 - protein, 41 aa, Artificial
  Triple agonist
  MISC_FEATURE (2)..(2): Xaa is aminoisobutyric acid (Aib)
  MISC_FEATURE (16)..(20): amino acids at positions 16 and 20 form a ring
YXQGTFTSDYSKYLDECRAKEFVQWLLAQKGKKNDWKHNIT

SEQ ID NO: 24 - protein, 39 aa, Artificial
  Triple agonist
  MISC_FEATURE (2)..(2): Xaa is aminoisobutyric acid (Aib)
  MISC_FEATURE (16)..(20): amino acids at positions 16 and 20 form a ring
YXQGTFTSDYSKYLDECRAKEFVQWLKNGGPSSGAPPPS

SEQ ID NO: 25 - protein, 39 aa, Artificial
  Triple agonist
  MISC_FEATURE (2)..(2): Xaa is aminoisobutyric acid (Aib)
HXQGTFTSDCSKYLDERAAQDFVQWLLDGGPSSGAPPPS

SEQ ID NO: 26 - protein, 39 aa, Artificial
  Triple agonist
  MISC_FEATURE (2)..(2): Xaa is aminoisobutyric acid (Aib)
HXQGTFTSDCSKYLDSRAAQDFVQWLLDGGPSSGAPPPS

SEQ ID NO: 27 - protein, 40 aa, Artificial
  Triple agonist
  MISC_FEATURE (2)..(2): Xaa is aminoisobutyric acid (Aib)
HXQGTFTSDYSKYLDERACQDFVQWLLDQGGPSSGAPPPS

SEQ ID NO: 28 - protein, 41 aa, Artificial
  Triple agonist
  MISC_FEATURE (2)..(2): Xaa is aminoisobutyric acid (Aib)
HXQGTFTSDYSKYLDEKRAQEFVCWLLAQKGKKNDWKHNIT

SEQ ID NO: 29 - protein, 30 aa, Artificial
  Triple agonist
  MISC_FEATURE (2)..(2): Xaa is aminoisobutyric acid (Aib)
  MISC_FEATURE (16)..(20): amino acids at positions 16 and 20 form a ring
HXQGTFTSDYSKYLDEKAAKEFVQWLLNTC

SEQ ID NO: 30 - protein, 30 aa, Artificial
  Triple agonist
  MISC_FEATURE (2)..(2): Xaa is aminoisobutyric acid (Aib)
  MISC_FEATURE (16)..(20): amino acids at positions 16 and 20 form a ring
HXQGTFTSDYSKYLDEKAQKEFVQWLLDTC

SEQ ID NO: 31 - protein, 29 aa, Artificial
  Triple agonist
  MISC_FEATURE (2)..(2): Xaa is aminoisobutyric acid (Aib)
  MISC_FEATURE (16)..(20): amino acids at positions 16 and 20 form a ring
HXQGTFTSDYSKYLDEKACKEFVQWLLAQ

SEQ ID NO: 32 - protein, 39 aa, Artificial
  Triple agonist
  MISC_FEATURE (2)..(2): Xaa is aminoisobutyric acid (Aib)
  MISC_FEATURE (16)..(20): amino acids at positions 16 and 20 form a ring
HXQGTFTSDYSKYLDEKACKDFVQWLLDGGPSSGAPPPS

SEQ ID NO: 33 - protein, 31 aa, Artificial
  Triple agonist
  MISC_FEATURE (2)..(2): Xaa is aminoisobutyric acid (Aib)
  MISC_FEATURE (16)..(20): amino acids at positions 16 and 20 form a ring
HXQGTFTSDYSIAMDEIHQKDFVNWLLAQKC

SEQ ID NO: 34 - protein, 31 aa, Artificial
  Triple agonist
  MISC_FEATURE (2)..(2): Xaa is aminoisobutyric acid (Aib)
  MISC_FEATURE (16)..(20): amino acids at positions 16 and 20 form a ring
HXQGTFTSDYSKYLDEKRQKEFVNWLLAQKC

SEQ ID NO: 35 - protein, 31 aa, Artificial
  Triple agonist
  MISC_FEATURE (2)..(2): Xaa is aminoisobutyric acid (Aib)
  MISC_FEATURE (16)..(20): amino acids at positions 16 and 20 form a ring
HXQGTFTSDYSIAMDEIHQKDFVNWLLNTKC

SEQ ID NO: 36 - protein, 40 aa, Artificial
  Triple agonist
  MISC_FEATURE (2)..(2): Xaa is aminoisobutyric acid (Aib)
  MISC_FEATURE (16)..(20): amino acids at positions 16 and 20 form a ring
HXQGTFTSDYSKYLCEKRQKEFVQWLLNGGPSSGAPPPSG

SEQ ID NO: 37 - protein, 40 aa, Artificial
  Triple agonist
  MISC_FEATURE (2)..(2): Xaa is aminoisobutyric acid (Aib)
  MISC_FEATURE (16)..(20): amino acids at positions 16 and 20 form a ring
HXQGTFTSDYSKYLDECRQKEFVQWLLNGGPSSGAPPPSG

SEQ ID NO: 38 - protein, 40 aa, Artificial
  Triple agonist
  MISC_FEATURE (1)..(1): Xaa is 4-imidazoacetyl (CA)
  MISC_FEATURE (2)..(2): Xaa is aminoisobutyric acid (Aib)
XXQGTFTSDKSSYLDERAAQDFVQWLLDGGPSSGAPPPSS

SEQ ID NO: 39 - protein, 40 aa, Artificial
  Triple agonist
  MISC_FEATURE (2)..(2): Xaa is aminoisobutyric acid (Aib)
HXQGTFTSDYSKYLDGQHAQCFVAWLLAGGGPSSGAPPPS

SEQ ID NO: 40 - protein, 39 aa, Artificial
  Triple agonist
  MISC_FEATURE (2)..(2): Xaa is aminoisobutyric acid (Aib)
HXQGTFTSDKSKYLDERACQDFVQWLLDGGPSSGAPPPS

SEQ ID NO: 41 - protein, 39 aa, Artificial
  Triple agonist
  MISC_FEATURE (2)..(2): Xaa is aminoisobutyric acid (Aib)
HXQGTFTSDKSKYLDECAAQDFVQWLLDGGPSSGAPPPS

SEQ ID NO: 42 - protein, 40 aa, Artificial
  Triple agonist
  MISC_FEATURE (2)..(2): Xaa is aminoisobutyric acid (Aib)
  MISC_FEATURE (16)..(20): amino acids at positions 16 and 20 form a ring
YXQGTFTSDYSKYLDEKRAKEFVQWLLDHHPSSGQPPPSC

SEQ ID NO: 43 - protein, 39 aa, Artificial
  Triple agonist
  MISC_FEATURE (2)..(2): Xaa is aminoisobutyric acid (Aib)
  MISC_FEATURE (16)..(20): amino acids at positions 16 and 20 form a ring
YXQGTFTSDYSKYLDEKRAKEFVQWLLDHHCSSGQPPPS

SEQ ID NO: 44 - protein, 39 aa, Artificial
  Triple agonist
HGQGTFTSDCSKQLDGQAAQEFVAWLLAGGPSSGAPPPS

SEQ ID NO: 45 - protein, 39 aa, Artificial
  Triple agonist
HGQGTFTSDCSKYMDGQAAQDFVAWLLAGGPSSGAPPPS

SEQ ID NO: 46 - protein, 39 aa, Artificial
  Triple agonist
HGQGTFTSDCSKYLDEQHAQEFVAWLLAGGPSSGAPPPS

SEQ ID NO: 47 - protein, 39 aa, Artificial
  Triple agonist
HGQGTFTSDCSKYLDGQRAQEFVAWLLAGGPSSGAPPPS

SEQ ID NO: 48 - protein, 39 aa, Artificial
  Triple agonist
HGQGTFTSDCSKYLDGQRAQDFVNWLLAGGPSSGAPPPS

SEQ ID NO: 49 - protein, 30 aa, Artificial
  Triple agonist
  MISC_FEATURE (1)..(1): Xaa is 4-imidazoacetyl (CA)
  MISC_FEATURE (2)..(2): Xaa is aminoisobutyric acid (Aib)
  MISC_FEATURE (16)..(20): amino acids at positions 16 and 20 form a ring
XXQGTFTSDYSICMDEIHQKDFVNWLLNTK

SEQ ID NO: 50 - protein, 40 aa, Artificial
  Triple agonist
  MISC_FEATURE (2)..(2): Xaa is aminoisobutyric acid (Aib)
  MISC_FEATURE (16)..(20): amino acids at positions 16 and 20 form a ring
HXQGTFTSDYSKYLDEKRAKEFVQWLLDHHPSSGQPPPSC

SEQ ID NO: 51 - protein, 30 aa, Artificial
  Triple agonist
  MISC_FEATURE (2)..(2): Xaa is aminoisobutyric acid (Aib)
  MISC_FEATURE (16)..(20): amino acids at positions 16 and 20 form a ring
HXQGTFTSDYSKYLDEKRQKEFVQWLLNTC

SEQ ID NO: 52 - protein, 30 aa, Artificial
  Triple agonist
  MISC_FEATURE (2)..(2): Xaa is aminoisobutyric acid (Aib)
  MISC_FEATURE (16)..(20): amino acids at positions 16 and 20 form a ring
HXQGTFTSDYSKYLDEKRQKEFVQWLLDTC

SEQ ID NO: 53 - protein, 30 aa, Artificial
  Triple agonist
  MISC_FEATURE (2)..(2): Xaa is aminoisobutyric acid (Aib)
  MISC_FEATURE (16)..(20): amino acids at positions 16 and 20 form a ring
HXEGTFTSDYSIAMDEIHQKDFVNWLLAQC

SEQ ID NO: 54 - protein, 30 aa, Artificial
  Triple agonist
  MISC_FEATURE (2)..(2): Xaa is aminoisobutyric acid (Aib)
  MISC_FEATURE (16)..(20): amino acids at positions 16 and 20 form a ring
HXEGTFTSDYSIAMDEIHQKDFVDWLLAEC

SEQ ID NO: 55 - protein, 30 aa, Artificial
  Triple agonist
  MISC_FEATURE (2)..(2): Xaa is aminoisobutyric acid (Aib)
  MISC_FEATURE (16)..(20): amino acids at positions 16 and 20 form a ring
HXQGTFTSDYSIAMDEIHQKDFVNWLLAQC

SEQ ID NO: 56 - protein, 30 aa, Artificial
  Triple agonist
  MISC_FEATURE (2)..(2): Xaa is aminoisobutyric acid (Aib)
  MISC_FEATURE (16)..(20): amino acids at positions 16 and 20 form a ring
HXQGTFTSDYSKYLDEKRQKEFVNWLLAQC

SEQ ID NO: 57 - protein, 30 aa, Artificial
  Triple agonist
  MISC_FEATURE (2)..(2): Xaa is aminoisobutyric acid (Aib)
  MISC_FEATURE (16)..(20): amino acids at positions 16 and 20 form a ring
HXQGTFTSDYSIAMDEIHQKDFVNWLLNTC

SEQ ID NO: 58 - protein, 31 aa, Artificial
  Triple agonist
  MISC_FEATURE (2)..(2): Xaa is aminoisobutyric acid (Aib)
  MISC_FEATURE (16)..(20): amino acids at positions 16 and 20 form a ring
HXQGTFTSDYSKYLDEKRQKEFVQWLLNTKC

SEQ ID NO: 59 - protein, 30 aa, Artificial
  Triple agonist
  MISC_FEATURE (1)..(1): Xaa is 4-imidazoacetyl (CA)
  MISC_FEATURE (2)..(2): Xaa is aminoisobutyric acid (Aib)
  MISC_FEATURE (16)..(20): amino acids at positions 16 and 20 form a ring
XXQGTFTSDYSICMDEKHQKDFVNWLLNTK

SEQ ID NO: 60 - protein, 30 aa, Artificial
  Triple agonist
  MISC_FEATURE (1)..(1): Xaa is 4-imidazoacetyl (CA)
  MISC_FEATURE (2)..(2): Xaa is aminoisobutyric acid (Aib)
  MISC_FEATURE (16)..(20): amino acids at positions 16 and 20 form a ring
XXQGTFTSDYSIAMDEKHCKDFVNWLLNTK

SEQ ID NO: 61 - protein, 30 aa, Artificial
  Triple agonist
  MISC_FEATURE (1)..(1): Xaa is 4-imidazoacetyl (CA)
  MISC_FEATURE (2)..(2): Xaa is aminoisobutyric acid (Aib)
  MISC_FEATURE (16)..(20): amino acids at positions 16 and 20 form a ring
XXQGTFTSDYSIAMDEIACKDFVNWLLNTK

SEQ ID NO: 62 - protein, 39 aa, Artificial
  Triple agonist
  MISC_FEATURE (1)..(1): Xaa is 4-imidazoacetyl (CA)
  MISC_FEATURE (2)..(2): Xaa is aminoisobutyric acid (Aib)
XXQGTFTSDKSKYLDERAAQDFVQWLLDGGPSSGAPPPS

SEQ ID NO: 63 - protein, 39 aa, Artificial
  Triple agonist
  MISC_FEATURE (1)..(1): Xaa is 4-imidazoacetyl (CA)
  MISC_FEATURE (2)..(2): Xaa is aminoisobutyric acid (Aib)
XXQGTFTSDCSKYLDERAAQDFVQWLLDGGPSSGAPPPS

SEQ ID NO: 64 - protein, 39 aa, Artificial
  Triple agonist
  MISC_FEATURE (2)..(2): Xaa is aminoisobutyric acid (Aib)
  MISC_FEATURE (16)..(20): amino acids at positions 16 and 20 form a ring
YXQGTFTSDYSKYLDECAAKEFVQWLLDHHPSSGQPPPS

SEQ ID NO: 65 - protein, 39 aa, Artificial
  Triple agonist
  MISC_FEATURE (2)..(2): Xaa is aminoisobutyric acid (Aib)
  MISC_FEATURE (16)..(20): amino acids at positions 16 and 20 form a ring
HXQGTFTSDYSKCLDEKRAKEFVQWLLDHHPSSGQPPPS

SEQ ID NO: 66 - protein, 39 aa, Artificial
  Triple agonist
  MISC_FEATURE (2)..(2): Xaa is aminoisobutyric acid (Aib)
  MISC_FEATURE (16)..(20): amino acids at positions 16 and 20 form a ring
YXQGTFTSDYSKYLDECRAKDFVQWLLDHHPSSGQPPPS

SEQ ID NO: 67 - protein, 39 aa, Artificial
  Triple agonist
  MISC_FEATURE (2)..(2): Xaa is aminoisobutyric acid (Aib)
  MISC_FEATURE (16)..(20): amino acids at positions 16 and 20 form a ring
YXQGTFTSDYSKYLDECAAKDFVQWLLDHHPSSGQPPPS

SEQ ID NO: 68 - protein, 39 aa, Artificial
  Triple agonist
  MISC_FEATURE (2)..(2): Xaa is aminoisobutyric acid (Aib)
  MISC_FEATURE (16)..(20): amino acids at positions 16 and 20 form a ring
YXQGTFTSDYSKCLDEKAAKEFVQWLLDHHPSSGQPPPS

SEQ ID NO: 69 - protein, 39 aa, Artificial
  Triple agonist
  MISC_FEATURE (2)..(2): Xaa is aminoisobutyric acid (Aib)
  MISC_FEATURE (16)..(20): amino acids at positions 16 and 20 form a ring
YXQGTFTSDYSKCLDERAAKEFVQWLLDHHPSSGQPPPS

SEQ ID NO: 70 - protein, 39 aa, Artificial
  Triple agonist
  MISC_FEATURE (2)..(2): Xaa is aminoisobutyric acid (Aib)
  MISC_FEATURE (16)..(20): amino acids at positions 16 and 20 form a ring
YXQGTFTSDYSKCLDEKRAKDFVQWLLDHHPSSGQPPPS

SEQ ID NO: 71 - protein, 39 aa, Artificial
  Triple agonist
  MISC_FEATURE (2)..(2): Xaa is aminoisobutyric acid (Aib)
  MISC_FEATURE (16)..(20): amino acids at positions 16 and 20 form a ring
YXQGTFTSDYSKYLDERACKDFVQWLLDHHPSSGQPPPS

SEQ ID NO: 72 - protein, 39 aa, Artificial
  Triple agonist
  MISC_FEATURE (2)..(2): Xaa is aminoisobutyric acid (Aib)
  MISC_FEATURE (16)..(20): amino acids at positions 16 and 20 form a ring
YXQGTFTSDCSKYLDERAAKDFVQWLLDHHPSSGQPPPS

SEQ ID NO: 73 - protein, 39 aa, Artificial
  Triple agonist
  MISC_FEATURE (1)..(1): Xaa is 4-imidazoacetyl (CA)
  MISC_FEATURE (2)..(2): Xaa is aminoisobutyric acid (Aib)
  MISC_FEATURE (16)..(20): amino acids at positions 16 and 20 form a ring
XXQGTFTSDYSKYLDECRAKEFVQWLLDHHPSSGQPPPS

SEQ ID NO: 74 - protein, 39 aa, Artificial
  Triple agonist
  MISC_FEATURE (1)..(1): Xaa is 4-imidazoacetyl (CA)
  MISC_FEATURE (2)..(2): Xaa is aminoisobutyric acid (Aib)
  MISC_FEATURE (16)..(20): amino acids at positions 16 and 20 form a ring
XXQGTFTSDYSKCLDEKRAKEFVQWLLDHHPSSGQPPPS

SEQ ID NO: 75 - protein, 40 aa, Artificial
  Triple agonist
  MISC_FEATURE (2)..(2): Xaa is aminoisobutyric acid (Aib)
  MISC_FEATURE (16)..(20): amino acids at positions 16 and 20 form a ring
YXQGTFTSDYSKYLDEKAAKEFVQWLLDHHPSSGQPPPSC

SEQ ID NO: 76 - protein, 40 aa, Artificial
  Triple agonist
  MISC_FEATURE (2)..(2): Xaa is aminoisobutyric acid (Aib)
  MISC_FEATURE (16)..(20): amino acids at positions 16 and 20 form a ring
YXQGTFTSDYSKYLDEKRAKDFVQWLLDHHPSSGQPPPSC

SEQ ID NO: 77 - protein, 40 aa, Artificial
  Triple agonist
  MISC_FEATURE (2)..(2): Xaa is aminoisobutyric acid (Aib)
  MISC_FEATURE (16)..(20): amino acids at positions 16 and 20 form a ring
YXQGTFTSDYSKYLDEKAAKDFVQWLLDHHPSSGQPPPSC

SEQ ID NO: 78 - protein, 31 aa, Artificial
  Triple agonist
  MISC_FEATURE (2)..(2): Xaa is aminoisobutyric acid (Aib)
  MISC_FEATURE (16)..(20): amino acids at positions 16 and 20 form a ring
HXQGTFTSDYSKYLDEKRQKEFVQWLLDTKC

SEQ ID NO: 79 - protein, 31 aa, Artificial
  Triple agonist
  MISC_FEATURE (2)..(2): Xaa is aminoisobutyric acid (Aib)
  MISC_FEATURE (16)..(20): amino acids at positions 16 and 20 form a ring
HXEGTFTSDYSIAMDEIHQKDFVNWLLAQKC

SEQ ID NO: 80 - protein, 31 aa, Artificial
  Triple agonist
  MISC_FEATURE (2)..(2): Xaa is aminoisobutyric acid (Aib)
  MISC_FEATURE (16)..(20): amino acids at positions 16 and 20 form a ring
HXEGTFTSDYSIAMDEIHQKDFVDWLLAEKC

SEQ ID NO: 81 - protein, 30 aa, Artificial
  Triple agonist
  MISC_FEATURE (1)..(1): Xaa is 4-imidazoacetyl (CA)
  MISC_FEATURE (2)..(2): Xaa is aminoisobutyric acid (Aib)
  MISC_FEATURE (16)..(20): amino acids at positions 16 and 20 form a ring
XXQGTFTSDYSKYLDEKRQKEFVQWLLNTC

SEQ ID NO: 82 - protein, 30 aa, Artificial
  Triple agonist
  MISC_FEATURE (1)..(1): Xaa is 4-imidazoacetyl (CA)
  MISC_FEATURE (2)..(2): Xaa is aminoisobutyric acid (Aib)
  MISC_FEATURE (16)..(20): amino acids at positions 16 and 20 form a ring
XXQGTFTSDYSKYLDEKRQKEFVQWLLDTC

SEQ ID NO: 83 - protein, 30 aa, Artificial
  Triple agonist
  MISC_FEATURE (1)..(1): Xaa is 4-imidazoacetyl (CA)
  MISC_FEATURE (2)..(2): Xaa is aminoisobutyric acid (Aib)
  MISC_FEATURE (16)..(20): amino acids at positions 16 and 20 form a ring
XXEGTFTSDYSIAMDEIHQKDFVNWLLAQC

SEQ ID NO: 84 - protein, 30 aa, Artificial
  Triple agonist
  MISC_FEATURE (1)..(1): Xaa is 4-imidazoacetyl (CA)
  MISC_FEATURE (2)..(2): Xaa is aminoisobutyric acid (Aib)
  MISC_FEATURE (16)..(20): amino acids at positions 16 and 20 form a ring
XXEGTFTSDYSIAMDEIHQKDFVDWLLAEC

SEQ ID NO: 85 - protein, 30 aa, Artificial
  Triple agonist
  MISC_FEATURE (1)..(1): Xaa is 4-imidazoacetyl (CA)
  MISC_FEATURE (2)..(2): Xaa is aminoisobutyric acid (Aib)
  MISC_FEATURE (16)..(20): amino acids at positions 16 and 20 form a ring
XXQGTFTSDYSIAMDEIHQKDFVNWLLAQC

SEQ ID NO: 86 - protein, 30 aa, Artificial
  Triple agonist
  MISC_FEATURE (1)..(1): Xaa is 4-imidazoacetyl (CA)
  MISC_FEATURE (2)..(2): Xaa is aminoisobutyric acid (Aib)
  MISC_FEATURE (16)..(20): amino acids at positions 16 and 20 form a ring
XXQGTFTSDYSKYLDEKRQKEFVNWLLAQC

SEQ ID NO: 87 - protein, 30 aa, Artificial
  Triple agonist
  MISC_FEATURE (1)..(1): Xaa is 4-imidazoacetyl (CA)
  MISC_FEATURE (2)..(2): Xaa is aminoisobutyric acid (Aib)
  MISC_FEATURE (16)..(20): amino acids at positions 16 and 20 form a ring
XXQGTFTSDYSIAMDEIHQKDFVNWLLNTC

SEQ ID NO: 88 - protein, 31 aa, Artificial
  Triple agonist
  MISC_FEATURE (1)..(1): Xaa is 4-imidazoacetyl (CA)
  MISC_FEATURE (2)..(2): Xaa is aminoisobutyric acid (Aib)
  MISC_FEATURE (16)..(20): amino acids at positions 16 and 20 form a ring
XXQGTFTSDYSKYLDEKRQKEFVQWLLNTKC

SEQ ID NO: 89 - protein, 31 aa, Artificial
  Triple agonist
  MISC_FEATURE (1)..(1): Xaa is 4-imidazoacetyl (CA)
  MISC_FEATURE (2)..(2): Xaa is aminoisobutyric acid (Aib)
  MISC_FEATURE (16)..(20): amino acids at positions 16 and 20 form a ring
XXQGTFTSDYSKYLDEKRQKEFVQWLLDTKC

SEQ ID NO: 90 - protein, 31 aa, Artificial
  Triple agonist
  MISC_FEATURE (1)..(1): Xaa is 4-imidazoacetyl (CA)
  MISC_FEATURE (2)..(2): Xaa is aminoisobutyric acid (Aib)
  MISC_FEATURE (16)..(20): amino acids at positions 16 and 20 form a ring
XXEGTFTSDYSIAMDEIHQKDFVNWLLAQKC

SEQ ID NO: 91 - protein, 31 aa, Artificial
  Triple agonist
  MISC_FEATURE (1)..(1): Xaa is 4-imidazoacetyl (CA)
  MISC_FEATURE (2)..(2): Xaa is aminoisobutyric acid (Aib)
  MISC_FEATURE (16)..(20): amino acids at positions 16 and 20 form a ring
XXEGTFTSDYSIAMDEIHQKDFVDWLLAEKC

SEQ ID NO: 92 - protein, 31 aa, Artificial
  Triple agonist
  MISC_FEATURE (1)..(1): Xaa is 4-imidazoacetyl (CA)
  MISC_FEATURE (2)..(2): Xaa is aminoisobutyric acid (Aib)
  MISC_FEATURE (16)..(20): amino acids at positions 16 and 20 form a ring
XXQGTFTSDYSIAMDEIHQKDFVNWLLAQKC

SEQ ID NO: 93 - protein, 31 aa, Artificial
  Triple agonist
  MISC_FEATURE (1)..(1): Xaa is 4-imidazoacetyl (CA)
  MISC_FEATURE (2)..(2): Xaa is aminoisobutyric acid (Aib)
  MISC_FEATURE (16)..(20): amino acids at positions 16 and 20 form a ring
XXQGTFTSDYSKYLDEKRQKEFVNWLLAQKC

SEQ ID NO: 94 - protein, 31 aa, Artificial
  Triple agonist
  MISC_FEATURE (1)..(1): Xaa is 4-imidazoacetyl (CA)
  MISC_FEATURE (2)..(2): Xaa is aminoisobutyric acid (Aib)
  MISC_FEATURE (16)..(20): amino acids at positions 16 and 20 form a ring
XXQGTFTSDYSIAMDEIHQKDFVNWLLNTKC

SEQ ID NO: 95 - protein, 39 aa, Artificial
  Triple agonist
  MISC_FEATURE (2)..(2): Xaa is aminoisobutyric acid (Aib)
  MISC_FEATURE (16)..(20): amino acids at positions 16 and 20 form a ring
YXQGTFTSDYSKYLDEKRAKEFVQWLLCHHPSSGQPPPS

SEQ ID NO: 96 - protein, 39 aa, Artificial
  Triple agonist
  MISC_FEATURE (2)..(2): Xaa is aminoisobutyric acid (Aib)
  MISC_FEATURE (16)..(20): amino acids at positions 16 and 20 form a ring
YXQGTFTSDYSKYLDEKRAKEFVQWLLDHCPSSGQPPPS

SEQ ID NO: 97 - protein, 39 aa, Artificial
  Triple agonist
  MISC_FEATURE (2)..(2): Xaa is aminoisobutyric acid (Aib)
  MISC_FEATURE (16)..(20): amino acids at positions 16 and 20 form a ring
YXQGTFTSDYSKYLDEKRAKEFVQWLLDCHPSSGQPPPS

SEQ ID NO: 98 - protein, 40 aa, Artificial
  Triple agonist
  MISC_FEATURE (2)..(2): Xaa is aminoisobutyric acid (Aib)
  MISC_FEATURE (16)..(20): amino acids at positions 16 and 20 form a ring
YXQGTFTSDYSKALDEKAAKEFVNWLLDHHPSSGQPPPSC

SEQ ID NO: 99 - protein, 40 aa, Artificial
  Triple agonist
  MISC_FEATURE (2)..(2): Xaa is aminoisobutyric acid (Aib)
  MISC_FEATURE (16)..(20): amino acids at positions 16 and 20 form a ring
YXQGTFTSDYSKALDEKAAKDFVNWLLDHHPSSGQPPPSC

SEQ ID NO: 100 - protein, 40 aa, Artificial
  Triple agonist
  MISC_FEATURE (2)..(2): Xaa is aminoisobutyric acid (Aib)
  MISC_FEATURE (16)..(20): amino acids at positions 16 and 20 form a ring
YXQGTFTSDYSKALDEKAAKEFVQWLLDQHPSSGQPPPSC

SEQ ID NO: 101 - protein, 40 aa, Artificial
  Triple agonist
  MISC_FEATURE (2)..(2): Xaa is aminoisobutyric acid (Aib)
  MISC_FEATURE (16)..(20): amino acids at positions 16 and 20 form a ring
YXQGTFTSDYSKALDEKAAKEFVNWLLDQHPSSGQPPPSC

SEQ ID NO: 102 - protein, 40 aa, Artificial
  Triple agonist
  MISC_FEATURE (2)..(2): Xaa is aminoisobutyric acid (Aib)
  MISC_FEATURE (16)..(20): amino acids at positions 16 and 20 form a ring
YXQGTFTSDYSKALDEKAAKDFVNWLLDQHPSSGQPPPSC

SEQ ID NO: 103 - protein, 30 aa, Artificial
  General Formula 1
  MISC_FEATURE (1)..(1): Xaa is His (H), 4-imidazoacetyl (CA), or Tyr (Y)
  MISC_FEATURE (2)..(2): Xaa is Gly (G), alpha-methyl-glutamic acid, or Aib (aminoisobutyric acid)
  MISC_FEATURE (3)..(3): Xaa is Glu (E) or Gln (Q)
  MISC_FEATURE (7)..(7): Xaa is Thr (T) or Ile (I)
  MISC_FEATURE (10)..(10): Xaa is Leu (L), Tyr (Y), Lys (K), Cys (C), or Val (V)
  MISC_FEATURE (12)..(12): Xaa is Lys (K), Ser (S), or Ile (I)
  MISC_FEATURE (13)..(13): Xaa is Gln (Q), Tyr (Y), Ala (A), or Cys (C)
  MISC_FEATURE (14)..(14): Xaa is Leu (L), Met (M), or Tyr (Y)
  MISC_FEATURE (15)..(15): Xaa is Cys (C), Asp (D), Glu (E), or Leu (L)
  MISC_FEATURE (16)..(16): Xaa is Gly (G), Glu (E), or Ser (S)
  MISC_FEATURE (17)..(17): Xaa is Gln (Q), Arg (R), Ile (I), Glu (E), Cys (C), or Lys (K)
  MISC_FEATURE (18)..(18): Xaa is Ala (A), Gln (Q), Arg (R), or His (H)
  MISC_FEATURE (19)..(19): Xaa is Ala (A), Gln (Q), Cys (C), or Val (V)
  MISC_FEATURE (20)..(20): Xaa is Lys (K), Gln (Q), or Arg (R)
  MISC_FEATURE (21)..(21): Xaa is Glu (E), Gln (Q), Leu (L), Cys (C), or Asp (D)
  MISC_FEATURE (23)..(23): Xaa is Ile (I) or Val (V)
  MISC_FEATURE (24)..(24): Xaa is Ala (A), Gln (Q), Cys (C), Asn (N), Asp (D), or Glu (E)
  MISC_FEATURE (27)..(27): Xaa is Val (V), Leu (L), Lys (K), or Met (M)
  MISC_FEATURE (28)..(28): Xaa is Cys (C), Lys (K), Ala (A), Asn (N), or Asp (D)
  MISC_FEATURE (29)..(29): Xaa is Cys (C), Gly (G), Gln (Q), Thr (T), Glu (E), or His (H)
  MISC_FEATURE (30)..(30): Xaa is Cys, Gly, Lys, or His, or is absent; and Xaa can be further linked to R1, wherein R1 is Cys, GKKNDWKHNIT, m-SSGAPPPS-n, or m-SSGQPPPS-n, or is absent, and wherein m is -Cys-, -Pro-, or -Gly-Pro-, and n is -Cys-, -Gly-, -Ser-, or
XXXGTFXSDXSXXXXXXXXXXFXXWLXXXX

SEQ ID NO: 104 - protein, 40 aa, Artificial
  General Formula 2
  MISC_FEATURE (1)..(1): Xaa is His (H), 4-imidazoacetyl (CA), or Tyr (Y)
  MISC_FEATURE (2)..(2): Xaa is Gly (G), alpha-methyl-glutamic acid, or Aib (aminoisobutyric acid)
  MISC_FEATURE (10)..(10): Xaa is Tyr (Y) or Cys (C)
  MISC_FEATURE (13)..(13): Xaa is Gln (Q), Tyr (Y), Ala (A), or Cys (C)
  MISC_FEATURE (14)..(14): Xaa is Leu (L), Met (M), or Tyr (Y)
  MISC_FEATURE (15)..(15): Xaa is Asp (D), Glu (E), or Leu (L)
  MISC_FEATURE (16)..(16): Xaa is Gly (G), Glu (E), or Ser (S)
  MISC_FEATURE (17)..(17): Xaa is Gln (Q), Arg (R), Ile (I), Glu (E), Cys (C), or Lys (K)
  MISC_FEATURE (18)..(18): Xaa is Ala (A), Gln (Q), Arg (R), or His (H)
  MISC_FEATURE (19)..(19): Xaa is Ala (A), Gln (Q), Cys (C), or Val (V)
  MISC_FEATURE (20)..(20): Xaa is Lys (K), Gln (Q), or Arg (R)
  MISC_FEATURE (21)..(21): Xaa is Glu (E), Gln (Q), Leu (L), Cys (C), or Asp (D)
  MISC_FEATURE (23)..(23): Xaa is Ile (I) or Val (V)
  MISC_FEATURE (24)..(24): Xaa is Ala (A), Gln (Q), Cys (C), Asn (N), or Glu (E)
  MISC_FEATURE (28)..(28): Xaa is Cys (C), Lys (K), Asn (N), or Asp (D)
  MISC_FEATURE (29)..(29): Xaa is Cys (C), Gly (G), Gln (Q), or His (H)
  MISC_FEATURE (30)..(30): Xaa is Cys (C), Gly (G), Lys (K), or His (H)
  MISC_FEATURE (31)..(31): Xaa is Pro (P) or Cys (C)
  MISC_FEATURE (40)..(40): Xaa is Cys (C), or is absent
XXQGTFTSDXSKXXXXXXXXXFXXWLLXXXXSSGQPPPSX

SEQ ID NO: 105 - protein, 40 aa, Artificial
  General Formula 3
  MISC_FEATURE (1)..(1): Xaa is His (H) or Tyr (Y)
  MISC_FEATURE (2)..(2): Xaa is alpha-methyl-glutamic acid, or Aib (aminoisobutyric acid)
  MISC_FEATURE (13)..(13): Xaa is Tyr (Y), Ala (A), or Cys (C)
  MISC_FEATURE (17)..(17): Xaa is Arg (R), Cys (C), or Lys (K)
  MISC_FEATURE (18)..(18): Xaa is Ala (A) or Arg (R)
  MISC_FEATURE (19)..(19): Xaa is Ala (A) or Cys (C)
  MISC_FEATURE (21)..(21): Xaa is Glu (E) or Asp (D)
  MISC_FEATURE (24)..(24): Xaa is Gln (Q) or Asn (N)
  MISC_FEATURE (28)..(28): Xaa is Cys (C) or Asp (D)
  MISC_FEATURE (29)..(29): Xaa is Cys (C), Gln (Q), or His (H)
  MISC_FEATURE (30)..(30): Xaa is Cys (C) or His (H)
  MISC_FEATURE (31)..(31): Xaa is Pro (P) or Cys (C)
  MISC_FEATURE (40)..(40): Xaa is Cys (C), or is absent
XXQGTFTSDYSKXLDEXXXKXFVXWLLXXXXSSGQPPPSX

SEQ ID NO: 106 - protein, 11 aa, Artificial
  R1
GKKNDWKHNIT

SEQ ID NO: 107 - protein, 8 aa, Artificial
  R1
SSGAPPPS

SEQ ID NO: 108 - protein, 8 aa, Artificial
  R1
SSGQPPPS

SEQ ID NO: 109 - protein, 9 aa, Artificial
  R1
CSSGQPPPS

SEQ ID NO: 110 - protein, 10 aa, Artificial
  R1
GPSSGAPPPS

SEQ ID NO: 111 - protein, 11 aa, Artificial
  R1
GPSSGAPPPSC

SEQ ID NO: 112 - protein, 9 aa, Artificial
  R1
PSSGAPPPS

SEQ ID NO: 113 - protein, 10 aa, Artificial
  R1
PSSGAPPPSG

SEQ ID NO: 114 - protein, 11 aa, Artificial
  R1
PSSGAPPPSHG

SEQ ID NO: 115 - protein, 10 aa, Artificial
  R1
PSSGAPPPSS

SEQ ID NO: 116 - protein, 9 aa, Artificial
  R1
PSSGQPPPS

SEQ ID NO: 117 - protein, 10 aa, Artificial
  R1
PSSGQPPPSC

SEQ ID NO: 118 - protein, 29 aa, Homo sapiens
HSQGTFTSDYSKYLDSRRAQDFVQWLMNT

SEQ ID NO: 119 - protein, 12 aa, Homo sapiens
ESKYGPPCPSCP

SEQ ID NO: 120 - protein, 11 aa, Artificial
  Variant of hinge region
ESKYGPPPSCP

SEQ ID NO: 121 - protein, 11 aa, Artificial
  Variant of hinge region
ESKYGPPCPSP

SEQ ID NO: 122 - protein, 10 aa, Artificial
  Variant of hinge region
ESKYGPPCPS

SEQ ID NO: 123 - protein, 10 aa, Artificial
  Variant of hinge region
ESKYGPPCPP

SEQ ID NO: 124 - protein, 8 aa, Artificial
  Variant of hinge region
KYGPPCPS

SEQ ID NO: 125 - protein, 8 aa, Artificial
  Variant of hinge region
ESKYGPPC

SEQ ID NO: 126 - protein, 7 aa, Artificial
  Variant of hinge region
EKYGPPC

SEQ ID NO: 127 - protein, 6 aa, Artificial
  Variant of hinge region
ESPSCP

SEQ ID NO: 128 - protein, 5 aa, Artificial
  Variant of hinge region
EPSCP

SEQ ID NO: 129 - protein, 4 aa, Artificial
  Variant of hinge region
PSCP

SEQ ID NO: 130 - protein, 10 aa, Artificial
  Variant of hinge region
ESKYGPPSCP

SEQ ID NO: 131 - protein, 9 aa, Artificial
  Variant of hinge region
KYGPPPSCP

SEQ ID NO: 132 - protein, 9 aa, Artificial
  Variant of hinge region
ESKYGPSCP

SEQ ID NO: 133 - protein, 8 aa, Artificial
  Variant of hinge region
ESKYGPPC

SEQ ID NO: 134 - protein, 7 aa, Artificial
  Variant of hinge region
KYGPPCP

SEQ ID NO: 135 - protein, 7 aa, Artificial
  Variant of hinge region
ESKPSCP

SEQ ID NO: 136 - protein, 6 aa, Artificial
  Variant of hinge region
ESPSCP

SEQ ID NO: 137 - protein, 4 aa, Artificial
  Variant of hinge region
EPSC

SEQ ID NO: 138 - protein, 3 aa, Artificial
  Variant of hinge region
SCP